European Patent Application EP 4 166 153 A1, published April 19, 2023. Title: HIGH REBAUDIOSIDE D-CONTENT STEVIA PLANT. Applicant: SUNTORY HOLDINGS LIMITED. The sequence listing filed with the application follows.

SEQUENCE LISTING (148 sequences)

SEQ ID NO: 1 - DNA, 203 bp, Stevia rebaudiana
aattatatgatagaaattgttttcacattttgtgtgccatacacgtcaacgcctctaagccacacgattaaggtatgacatttagaataaaatcttttattattggaagatagagacaaaatcttttctttccttatttattttttataataattacacgcatcttctattctcaactactttaacctatatgcgctagtcca

SEQ ID NO: 2 - DNA, 364 bp, Stevia rebaudiana
gaaactgaaagagaagtaagataacagaatgcgtttyttcgtaaataatcttttcttttatttttatcttcaaaaaataaataaccaagatttgtttggatttgtttctatttatttagacaaatcattattaatatttaatmtttcyccgtgaattatatgatagaaattgttttcacattttgtgtgccayacacgtcaacgcctctaagccacacgattaaggtatgacatttagaataaaatcttttattattggaagatagagacaaaatcttttctttccttatttattttttataataattacacgcatcttctattctcaactactttaacctatatgcgctagtccactacgtag

SEQ ID NO: 3 - DNA, 202 bp, Stevia rebaudiana
agagaagtaagwtaacagaatgcgtttcttcgtaaataatcttttcttttatttttatcttcaaaaaataaataaccaagatttgtttggatttgtttctatttatttagacaaatcattattaatatttaatmtttcyccgtgaattatatgatagaaattgttttcacattttgtgtgccayacacgtcaacgcctctaa

SEQ ID NO: 4 - DNA, 137 bp, Stevia rebaudiana
ccaagatttgtttggatttgtttctatttatttagacaaatcattattaatatttaatatttcyccgtgaattatatgatagaaattgttttcacattttgtgtgccayacacgtcaacgcctctaagccacacgat

SEQ ID NO: 5 - DNA, 137 bp, Stevia rebaudiana
ccaagatttgtttggatttgtttctatttatttagacaaatcattattaatatttaatmtttccccgtgaattatatgatagaaattgttttcacattttgtgtgccayacacgtcaacgcctctaagccacacgat

SEQ ID NO: 6 - DNA, 326 bp, Stevia rebaudiana
ggcagccattgatgatgttgttgaatgtgattaatttgaatgttataaagaatttggaaaagaaaaaggaggggacaaagttgatgaaattaggggagttatgattatgatggccatggtgattgtgatgagtggcactatgtaatctaatatttgaagatatgagaccacttgaccatgttataatcttatacaaaataattaatccctcacggtaatttttttctaatccttaaactgaaatttgaaagtaatttgagatagtgtttcccctaatttatgcttttagtatgcatttattctatcatattttctatgagaattgg

SEQ ID NO: 7 - DNA, 70 bp, Stevia rebaudiana
tgattttgaaaggatctgactgtatgtttataagacatagttatgagtttgaaccccaatggctaaccct

SEQ ID NO: 8 - DNA, 39 bp, Artificial Sequence
  Synthetic DNA
aattatatgatagaaattgttttcacattttgtgtgcca

SEQ ID NO: 9 - DNA, 26 bp, Artificial Sequence
  Synthetic DNA
tggactagcgcatataggttaaagta

SEQ ID NO: 10 - DNA, 20 bp, Artificial Sequence
  Synthetic DNA
gaaactgaaagagaagtaag

SEQ ID NO: 11 - DNA, 20 bp, Artificial Sequence
  Synthetic DNA
ctacgtagtggactagcgca

SEQ ID NO: 12 - DNA, 24 bp, Artificial Sequence
  Synthetic DNA
agagaagtaagwtaacagaatgcg

SEQ ID NO: 13 - DNA, 20 bp, Artificial Sequence
  Synthetic DNA
ttagaggcgttgacgtgtrt

SEQ ID NO: 14 - DNA, 25 bp, Artificial Sequence
  Synthetic DNA
ccaagatttgtttggatttgtttct

SEQ ID NO: 15 - DNA, 19 bp, Artificial Sequence
  Synthetic DNA
atcgtgtggcttagaggcg

SEQ ID NO: 16 - DNA, 25 bp, Artificial Sequence
  Synthetic DNA
ccaagatttgtttggatttgtttct

SEQ ID NO: 17 - DNA, 19 bp, Artificial Sequence
  Synthetic DNA
atcgtgtggcttagaggcg

SEQ ID NO: 18 - DNA, 25 bp, Artificial Sequence
  Synthetic DNA
ggcagccattgatgatgttgttgaa

SEQ ID NO: 19 - DNA, 36 bp, Artificial Sequence
  Synthetic DNA
ccaattctcatagaaaatatgatagaataaatgcat

SEQ ID NO: 20 - DNA, 32 bp, Artificial Sequence
  Synthetic DNA
tgattttgaaaggatctgactgtatgtttata

SEQ ID NO: 21 - DNA, 20 bp, Artificial Sequence
  Synthetic DNA
agggttagccattggggttc

SEQ ID NO: 22 - DNA, 203 bp, Stevia rebaudiana
aattatatgatagaaattgttttcacattttgtgtgccacacacgtcaacgcctctaagccacacgattaaggtatgacatttagaataaaatcttttattattggaagatagagacaaaatcttttctttccttatttattttttataataattacacgcatcttctattctcaactactttaacctatatgcgctagtcca

SEQ ID NO: 23 - DNA, 21 bp, Stevia rebaudiana
ttgtgtgccacacacgtcaac

SEQ ID NO: 24 - DNA, 41 bp, Stevia rebaudiana
ttttcacattttgtgtgccacacacgtcaacgcctctaagc

SEQ ID NO: 25 - DNA, 61 bp, Stevia rebaudiana
atagaaattgttttcacattttgtgtgccacacacgtcaacgcctctaagccacacgatta

SEQ ID NO: 26 - DNA, 364 bp, Stevia rebaudiana
gaaactgaaagagaagtaagttaacagaatgcgtttyttcgtaaataatcttttcttttatttttatcttcaaaaaataaataaccaagatttgtttggatttgtttctatttatttagacaaatcattattaatatttaatmtttcyccgtgaattatatgatagaaattgttttcacattttgtgtgccayacacgtcaacgcctctaagccacacgattaaggtatgacatttagaataaaatcttttattattggaagatagagacaaaatcttttctttccttatttattttttataataattacacgcatcttctattctcaactactttaacctatatgcgctagtccactacgtag

SEQ ID NO: 27 - DNA, 21 bp, Stevia rebaudiana
gagaagtaagttaacagaatg

SEQ ID NO: 28 - DNA, 41 bp, Stevia rebaudiana
gaaactgaaagagaagtaagttaacagaatgcgtttyttcg

SEQ ID NO: 29 - DNA, 61 bp, Stevia rebaudiana
aatgtttaaggaaactgaaagagaagtaagttaacagaatgcgtttyttcgtaaataatct

SEQ ID NO: 30 - DNA, 202 bp, Stevia rebaudiana
agagaagtaagwtaacagaatgcgttttttcgtaaataatcttttcttttatttttatcttcaaaaaataaataaccaagatttgtttggatttgtttctatttatttagacaaatcattattaatatttaatmtttcyccgtgaattatatgatagaaattgttttcacattttgtgtgccayacacgtcaacgcctctaa

SEQ ID NO: 31 - DNA, 21 bp, Stevia rebaudiana
gaatgcgttttttcgtaaata

SEQ ID NO: 32 - DNA, 41 bp, Stevia rebaudiana
taagwtaacagaatgcgttttttcgtaaataatcttttctt

SEQ ID NO: 33 - DNA, 61 bp, Stevia rebaudiana
gaaagagaagtaagwtaacagaatgcgttttttcgtaaataatcttttcttttatttttat

SEQ ID NO: 34 - DNA, 137 bp, Stevia rebaudiana
ccaagatttgtttggatttgtttctatttatttagacaaatcattattaatatttaatctttcyccgtgaattatatgatagaaattgttttcacattttgtgtgccayacacgtcaacgcctctaagccacacgat

SEQ ID NO: 35 - DNA, 21 bp, Stevia rebaudiana
aatatttaatctttcyccgtg

SEQ ID NO: 36 - DNA, 41 bp, Stevia rebaudiana
aatcattattaatatttaatctttcyccgtgaattatatga

SEQ ID NO: 37 - DNA, 61 bp, Stevia rebaudiana
tatttagacaaatcattattaatatttaatctttcyccgtgaattatatgatagaaattgt

SEQ ID NO: 38 - DNA, 137 bp, Stevia rebaudiana
ccaagatttgtttggatttgtttctatttatttagacaaatcattattaatatttaatmtttctccgtgaattatatgatagaaattgttttcacattttgtgtgccayacacgtcaacgcctctaagccacacgat

SEQ ID NO: 39 - DNA, 21 bp, Stevia rebaudiana
ttaatmtttctccgtgaatta

SEQ ID NO: 40 - DNA, 41 bp, Stevia rebaudiana
ttattaatatttaatmtttctccgtgaattatatgatagaa

SEQ ID NO: 41 - DNA, 61 bp, Stevia rebaudiana
agacaaatcattattaatatttaatmtttctccgtgaattatatgatagaaattgttttca

SEQ ID NO: 42 - DNA, 326 bp, Stevia rebaudiana
ggcagccattgatgatgttgttgaatgtgattaatttgaatgttataaagaatttggaaaagaaaaaggaggggacaaagttgatgaaattaggggagttatgattatgatggccatggtgattgtgatgagtggcactatgtaatctaatatttgaagatatgagaccacttgaccatgttataatcttatacaaaataattaatccctcacggtaatttttttctaatccttaaactgaaatttgaaagtaatttgagatagtgtttcccctaatttatgcttttagcatgcatttattctatcatattttctatgagaattgg

SEQ ID NO: 43 - DNA, 21 bp, Stevia rebaudiana
atgcttttagcatgcatttat

SEQ ID NO: 44 - DNA, 41 bp, Stevia rebaudiana
cccctaatttatgcttttagcatgcatttattctatcatat

SEQ ID NO: 45 - DNA, 61 bp, Stevia rebaudiana
gatagtgtttcccctaatttatgcttttagcatgcatttattctatcatattttctatgag

SEQ ID NO: 46 - DNA, 70 bp, Stevia rebaudiana
tgattttgaaaggatctgactgtatgtttatatgacatagttatgagtttgaaccccaatggctaaccct

SEQ ID NO: 47 - DNA, 21 bp, Stevia rebaudiana
tatgtttatatgacatagtta

SEQ ID NO: 48 - DNA, 41 bp, Stevia rebaudiana
gatctgactgtatgtttatatgacatagttatgagtttgaa

SEQ ID NO: 49 - DNA, 61 bp, Stevia rebaudiana
attttgaaaggatctgactgtatgtttatatgacatagttatgagtttgaaccccaatggc

SEQ ID NO: 50 - DNA, 39 bp, Artificial Sequence
  Synthetic DNA
aattatatgatagaaattgttttcacattttgtgtgccg

SEQ ID NO: 51 - DNA, 26 bp, Artificial Sequence
  Synthetic DNA
tggactagcgcatataggttaaagta

SEQ ID NO: 52 - DNA, 203 bp, Artificial Sequence
  Synthetic DNA
aattatatgatagaaattgttttcacattttgtgtgccgcacacgtcaacgcctctaagccacacgattaaggtatgacatttagaataaaatcttttattattggaagatagagacaaaatcttttctttccttatttattttttataataattacacgcatcttctattctcaactactttaacctatatgcgctagtcca

SEQ ID NO: 53 - DNA, 203 bp, Artificial Sequence
  Synthetic DNA
aattatatgatagaaattgttttcacattttgtgtgccgtacacgtcaacgcctctaagccacacgattaaggtatgacatttagaataaaatcttttattattggaagatagagacaaaatcttttctttccttatttattttttataataattacacgcatcttctattctcaactactttaacctatatgcgctagtcca

SEQ ID NO: 54 - DNA, 40 bp, Artificial Sequence
  Synthetic DNA
aattatatgatagaaattgttttcacattttgtgtgccgt

SEQ ID NO: 55 - DNA, 163 bp, Artificial Sequence
  Synthetic DNA
acacgtcaacgcctctaagccacacgattaaggtatgacatttagaataaaatcttttattattggaagatagagacaaaatcttttctttccttatttattttttataataattacacgcatcttctattctcaactactttaacctatatgcgctagtcca

SEQ ID NO: 56 - DNA, 20 bp, Artificial Sequence
  Synthetic DNA
gaaactgaaagagaagaacg

SEQ ID NO: 57 - DNA, 20 bp, Artificial Sequence
  Synthetic DNA
ctacgtagtggactagcgca

SEQ ID NO: 58 - DNA, 364 bp, Artificial Sequence
  Synthetic DNA
gaaactgaaagagaagaacgttaacagaatgcgtttyttcgtaaataatcttttcttttatttttatcttcaaaaaataaataaccaagatttgtttggatttgtttctatttatttagacaaatcattattaatatttaatmtttcyccgtgaattatatgatagaaattgttttcacattttgtgtgccayacacgtcaacgcctctaagccacacgattaaggtatgacatttagaataaaatcttttattattggaagatagagacaaaatcttttctttccttatttattttttataataattacacgcatcttctattctcaactactttaacctatatgcgctagtccactacgtag

SEQ ID NO: 59 - DNA, 364 bp, Artificial Sequence
  Synthetic DNA
gaaactgaaagagaagaacgataacagaatgcgtttyttcgtaaataatcttttcttttatttttatcttcaaaaaataaataaccaagatttgtttggatttgtttctatttatttagacaaatcattattaatatttaatmtttcyccgtgaattatatgatagaaattgttttcacattttgtgtgccayacacgtcaacgcctctaagccacacgattaaggtatgacatttagaataaaatcttttattattggaagatagagacaaaatcttttctttccttatttattttttataataattacacgcatcttctattctcaactactttaacctatatgcgctagtccactacgtag

SEQ ID NO: 60 - DNA, 18 bp, Artificial Sequence
  Synthetic DNA
gaaactgaaagagaagaa

SEQ ID NO: 61 - DNA, 346 bp, Artificial Sequence
  Synthetic DNA
cgttaacagaatgcgtttyttcgtaaataatcttttcttttatttttatcttcaaaaaataaataaccaagatttgtttggatttgtttctatttatttagacaaatcattattaatatttaatmtttcyccgtgaattatatgatagaaattgttttcacattttgtgtgccayacacgtcaacgcctctaagccacacgattaaggtatgacatttagaataaaatcttttattattggaagatagagacaaaatcttttctttccttatttattttttataataattacacgcatcttctattctcaactactttaacctatatgcgctagtccactacgtag

SEQ ID NO: 62 - DNA, 20 bp, Artificial Sequence
  Synthetic DNA
taagwtaacagaatgcgagc

SEQ ID NO: 63 - DNA, 20 bp, Artificial Sequence
  Synthetic DNA
acgtagtggactagcgcata

SEQ ID NO: 64 - DNA, 353 bp, Artificial Sequence
  Synthetic DNA
taagwtaacagaatgcgagctttcgtaaataatcttttcttttatttttatcttcaaaaaataaataaccaagatttgtttggatttgtttctatttatttagacaaatcattattaatatttaatmtttcyccgtgaattatatgatagaaattgttttcacattttgtgtgccayacacgtcaacgcctctaagccacacgattaaggtatgacatttagaataaaatcttttattattggaagatagagacaaaatcttttctttccttatttattttttataataattacacgcatcttctattctcaactactttaacctatatgcgctatgcgctagtccactacgt

SEQ ID NO: 65 - DNA, 353 bp, Artificial Sequence
  Synthetic DNA
taagwtaacagaatgcgagccttcgtaaataatcttttcttttatttttatcttcaaaaaataaataaccaagatttgtttggatttgtttctatttatttagacaaatcattattaatatttaatmtttcyccgtgaattatatgatagaaattgttttcacattttgtgtgccayacacgtcaacgcctctaagccacacgattaaggtatgacatttagaataaaatcttttattattggaagatagagacaaaatcttttctttccttatttattttttataataattacacgcatcttctattctcaactactttaacctatatgcgctatgcgctagtccactacgt

SEQ ID NO: 66 - DNA, 19 bp, Artificial Sequence
  Synthetic DNA
taagwtaacagaatgcgag

SEQ ID NO: 67 - DNA, 334 bp, Artificial Sequence
  Synthetic DNA
ctttcgtaaataatcttttcttttatttttatcttcaaaaaataaataaccaagatttgtttggatttgtttctatttatttagacaaatcattattaatatttaatmtttcyccgtgaattatatgatagaaattgttttcacattttgtgtgccayacacgtcaacgcctctaagccacacgattaaggtatgacatttagaataaaatcttttattattggaagatagagacaaaatcttttctttccttatttattttttataataattacacgcatcttctattctcaactactttaacctatatgcgctatgcgctagtccactacgt

SEQ ID NO: 68 - DNA, 21 bp, Artificial Sequence
  Synthetic DNA
aaatcattattaatatttaag

SEQ ID NO: 69 - DNA, 20 bp, Artificial Sequence
  Synthetic DNA
tggcgccggcgaacggttgt

SEQ ID NO: 70 - DNA, 349 bp, Artificial Sequence
  Synthetic DNA
aaatcattattaatatttaagctttcyccgtgaattatatgatagaaattgttttcacattttgtgtgccayacacgtcaacgcctctaagccacacgattaaggtatgacatttagaataaaatcttttattattggaagatagagacaaaatcttttctttccttatttattttttataataattacacgcatcttctattctcaactactttaacctatatgcgctagtccactacgtagagtcgttcattctgttttcgagtttctacgttcattctgtttttgagtgtaaacatcagtcaaatcccatggaaaataaaacggagacaaccgttcgccggcgcca

SEQ ID NO: 71 - DNA, 349 bp, Artificial Sequence
  Synthetic DNA
aaatcattattaatatttaagatttcyccgtgaattatatgatagaaattgttttcacattttgtgtgccayacacgtcaacgcctctaagccacacgattaaggtatgacatttagaataaaatcttttattattggaagatagagacaaaatcttttctttccttatttattttttataataattacacgcatcttctattctcaactactttaacctatatgcgctagtccactacgtagagtcgttcattctgttttcgagtttctacgttcattctgtttttgagtgtaaacatcagtcaaatcccatggaaaataaaacggagacaaccgttcgccggcgcca

SEQ ID NO: 72 - DNA, 21 bp, Artificial Sequence
  Synthetic DNA
aaatcattattaatatttaag

SEQ ID NO: 73 - DNA, 328 bp, Artificial Sequence
  Synthetic DNA
ctttcyccgtgaattatatgatagaaattgttttcacattttgtgtgccayacacgtcaacgcctctaagccacacgattaaggtatgacatttagaataaaatcttttattattggaagatagagacaaaatcttttctttccttatttattttttataataattacacgcatcttctattctcaactactttaacctatatgcgctagtccactacgtagagtcgttcattctgttttcgagtttctacgttcattctgtttttgagtgtaaacatcagtcaaatcccatggaaaataaaacggagacaaccgttcgccggcgcca

SEQ ID NO: 74 - DNA, 22 bp, Artificial Sequence
  Synthetic DNA
cattattaatatttaatmtagc

SEQ ID NO: 75 - DNA, 20 bp, Artificial Sequence
  Synthetic DNA
tctctggcgccggcgaacgg

SEQ ID NO: 76 - DNA, 349 bp, Artificial Sequence
  Synthetic DNA
cattattaatatttaatmtagctccgtgaattatatgatagaaattgttttcacattttgtgtgccayacacgtcaacgcctctaagccacacgattaaggtatgacatttagaataaaatcttttattattggaagatagagacaaaatcttttctttccttatttattttttataataattacacgcatcttctattctcaactactttaacctatatgcgctagtccactacgtagagtcgttcattctgttttcgagtttctacgttcattctgtttttgagtgtaaacatcagtcaaatcccatggaaaataaaacggagacaaccgttcgccggcgccagaga

SEQ ID NO: 77 - DNA, 349 bp, Artificial Sequence
  Synthetic DNA
cattattaatatttaatmtagccccgtgaattatatgatagaaattgttttcacattttgtgtgccayacacgtcaacgcctctaagccacacgattaaggtatgacatttagaataaaatcttttattattggaagatagagacaaaatcttttctttccttatttattttttataataattacacgcatcttctattctcaactactttaacctatatgcgctagtccactacgtagagtcgttcattctgttttcgagtttctacgttcattctgtttttgagtgtaaacatcagtcaaatcccatggaaaataaaacggagacaaccgttcgccggcgccagaga

SEQ ID NO: 78 - DNA, 21 bp, Artificial Sequence
  Synthetic DNA
cattattaatatttaatmtag

SEQ ID NO: 79 - DNA, 328 bp, Artificial Sequence
  Synthetic DNA
ctccgtgaattatatgatagaaattgttttcacattttgtgtgccayacacgtcaacgcctctaagccacacgattaaggtatgacatttagaataaaatcttttattattggaagatagagacaaaatcttttctttccttatttattttttataataattacacgcatcttctattctcaactactttaacctatatgcgctagtccactacgtagagtcgttcattctgttttcgagtttctacgttcattctgtttttgagtgtaaacatcagtcaaatcccatggaaaataaaacggagacaaccgttcgccggcgccagaga

SEQ ID NO: 80 - DNA, 25 bp, Artificial Sequence
  Synthetic DNA
ggcagccattgatgatgttgttgaa

SEQ ID NO: 81 - DNA, 36 bp, Artificial Sequence
  Synthetic DNA
ccaattctcatagaaaatatgatagaataaatgcgt

SEQ ID NO: 82 - DNA, 326 bp, Artificial Sequence
  Synthetic DNA
ggcagccattgatgatgttgttgaatgtgattaatttgaatgttataaagaatttggaaaagaaaaaggaggggacaaagttgatgaaattaggggagttatgattatgatggccatggtgattgtgatgagtggcactatgtaatctaatatttgaagatatgagaccacttgaccatgttataatcttatacaaaataattaatccctcacggtaatttttttctaatccttaaactgaaatttgaaagtaatttgagatagtgtttcccctaatttatgcttttagcacgcatttattctatcatattttctatgagaattgg

SEQ ID NO: 83 - DNA, 326 bp, Artificial Sequence
  Synthetic DNA
ggcagccattgatgatgttgttgaatgtgattaatttgaatgttataaagaatttggaaaagaaaaaggaggggacaaagttgatgaaattaggggagttatgattatgatggccatggtgattgtgatgagtggcactatgtaatctaatatttgaagatatgagaccacttgaccatgttataatcttatacaaaataattaatccctcacggtaatttttttctaatccttaaactgaaatttgaaagtaatttgagatagtgtttcccctaatttatgcttttagtacgcatttattctatcatattttctatgagaattgg

SEQ ID NO: 84 - DNA, 290 bp, Artificial Sequence
  Synthetic DNA
ggcagccattgatgatgttgttgaatgtgattaatttgaatgttataaagaatttggaaaagaaaaaggaggggacaaagttgatgaaattaggggagttatgattatgatggccatggtgattgtgatgagtggcactatgtaatctaatatttgaagatatgagaccacttgaccatgttataatcttatacaaaataattaatccctcacggtaatttttttctaatccttaaactgaaatttgaaagtaatttgagatagtgtttcccctaatttatgcttttagt

SEQ ID NO: 85 - DNA, 36 bp, Artificial Sequence
  Synthetic DNA
acgcatttattctatcatattttctatgagaattgg

SEQ ID NO: 86 - DNA, 32 bp, Artificial Sequence
  Synthetic DNA
tgattttgaaaggatctgactgtatgttttta

SEQ ID NO: 87 - DNA, 20 bp, Artificial Sequence
  Synthetic DNA
tgttgaccatcaagccacat

SEQ ID NO: 88 - DNA, 196 bp, Artificial Sequence
  Synthetic DNA
tgattttgaaaggatctgactgtatgtttttatgacatagttatgagtttgaaccccaatggctaacccttttagagaagctccatcacctaccggtggttcctgtcggattattgccaccagaaaaacccaccaacatcgaagacgggaatgatgagacgtgggacacagtcaagatgtggcttgatggtcaaca

SEQ ID NO: 89 - DNA, 196 bp, Artificial Sequence
  Synthetic DNA
tgattttgaaaggatctgactgtatgtttttaagacatagttatgagtttgaaccccaatggctaacccttttagagaagctccatcacctaccggtggttcctgtcggattattgccaccagaaaaacccaccaacatcgaagacgggaatgatgagacgtgggacacagtcaagatgtggcttgatggtcaaca

SEQ ID NO: 90 - DNA, 30 bp, Artificial Sequence
  Synthetic DNA
tgattttgaaaggatctgactgtatgtttt

SEQ ID NO: 91 - DNA, 166 bp, Artificial Sequence
  Synthetic DNA
taagacatagttatgagtttgaaccccaatggctaacccttttagagaagctccatcacctaccggtggttcctgtcggattattgccaccagaaaaacccaccaacatcgaagacgggaatgatgagacgtgggacacagtcaagatgtggcttgatggtcaaca

SEQ ID NO: 92 - DNA, 21 bp, Stevia rebaudiana
ttgtgtgccatacacgtcaac

SEQ ID NO: 93 - DNA, 41 bp, Stevia rebaudiana
ttttcacattttgtgtgccatacacgtcaacgcctctaagc

SEQ ID NO: 94 - DNA, 61 bp, Stevia rebaudiana
atagaaattgttttcacattttgtgtgccatacacgtcaacgcctctaagccacacgatta

SEQ ID NO: 95 - DNA, 21 bp, Stevia rebaudiana
gagaagtaagataacagaatg

SEQ ID NO: 96 - DNA, 41 bp, Stevia rebaudiana
gaaactgaaagagaagtaagataacagaatgcgtttyttcg

SEQ ID NO: 97 - DNA, 61 bp, Stevia rebaudiana
aatgtttaaggaaactgaaagagaagtaagataacagaatgcgtttyttcgtaaataatct

SEQ ID NO: 98 - DNA, 21 bp, Stevia rebaudiana
gaatgcgtttcttcgtaaata

SEQ ID NO: 99 - DNA, 41 bp, Stevia rebaudiana
taagwtaacagaatgcgtttcttcgtaaataatcttttctt

SEQ ID NO: 100 - DNA, 61 bp, Stevia rebaudiana
gaaagagaagtaagwtaacagaatgcgtttcttcgtaaataatcttttcttttatttttat

SEQ ID NO: 101 - DNA, 21 bp, Stevia rebaudiana
aatatttaatatttcyccgtg

SEQ ID NO: 102 - DNA, 41 bp, Stevia rebaudiana
aatcattattaatatttaatatttcyccgtgaattatatga

SEQ ID NO: 103 - DNA, 61 bp, Stevia rebaudiana
tatttagacaaatcattattaatatttaatatttcyccgtgaattatatgatagaaattgt

SEQ ID NO: 104 - DNA, 21 bp, Stevia rebaudiana
ttaatmtttccccgtgaatta

SEQ ID NO: 105 - DNA, 41 bp, Stevia rebaudiana
ttattaatatttaatmtttccccgtgaattatatgatagaa

SEQ ID NO: 106 - DNA, 61 bp, Stevia rebaudiana
agacaaatcattattaatatttaatmtttccccgtgaattatatgatagaaattgttttca

SEQ ID NO: 107 - DNA, 21 bp, Stevia rebaudiana
atgcttttagtatgcatttat

SEQ ID NO: 108 - DNA, 41 bp, Stevia rebaudiana
cccctaatttatgcttttagtatgcatttattctatcatat

SEQ ID NO: 109 - DNA, 61 bp, Stevia rebaudiana
gatagtgtttcccctaatttatgcttttagtatgcatttattctatcatattttctatgag

SEQ ID NO: 110 - DNA, 21 bp, Stevia rebaudiana
tatgtttataagacatagtta

SEQ ID NO: 111 - DNA, 41 bp, Stevia rebaudiana
gatctgactgtatgtttataagacatagttatgagtttgaa

SEQ ID NO: 112 - DNA, 61 bp, Stevia rebaudiana
attttgaaaggatctgactgtatgtttataagacatagttatgagtttgaaccccaatggc

SEQ ID NO: 113 - DNA, 20 bp, Artificial Sequence
  Synthetic DNA
ttttcacattttgtgtgtca

SEQ ID NO: 114 - DNA, 20 bp, Artificial Sequence
  Synthetic DNA
ttttcacattttgtgtgccg

SEQ ID NO: 115 - DNA, 340 bp, Artificial Sequence
  Synthetic DNA
ttttcacattttgtgtgccatacacgtcaacgcctctaagccacacgattaaggtatgacatttagaataaaatcttttattattggaagatagagacaaaatcttttctttccttatttattttttataataattacacgcatcttctattctcaactactttaacctatatgcgctagtccactacgtagagtcgttcattctgttttcgagtttctacgttcattctgtttttgagtgtaaacatcagtcaaatcccatggaaaataaaacggagacaaccgttcgccggcgccagagaataatattgttcccggtaccatttcaaggccacataag

SEQ ID NO: 116 - DNA, 340 bp, Artificial Sequence
  Synthetic DNA
ttttcacattttgtgtgccacacacgtcaacgcctctaagccacacgattaaggtatgacatttagaataaaatcttttattattggaagatagagacaaaatcttttctttccttatttattttttataataattacacgcatcttctattctcaactactttaacctatatgcgctagtccactacgtagagtcgttcattctgttttcgagtttctacgttcattctgtttttgagtgtaaacatcagtcaaatcccatggaaaataaaacggagacaaccgttcgccggcgccagagaataatattgttcccggtaccatttcaaggccacataag

SEQ ID NO: 117 - DNA, 21 bp, Artificial Sequence
  Synthetic DNA
cttatgtggccttgaaatggt

SEQ ID NO: 118 - DNA, 20 bp, Artificial Sequence
  Synthetic DNA
gaaactgaaagagaagtagc

SEQ ID NO: 119 - DNA, 20 bp, Artificial Sequence
  Synthetic DNA
gaaactgaaagagaagttaa

SEQ ID NO: 120 - DNA, 20 bp, Artificial Sequence
  Synthetic DNA
taagwtaacagaatgagatc

SEQ ID NO: 121 - DNA, 20 bp, Artificial Sequence
  Synthetic DNA
taagwtaacagaatgagtac

SEQ ID NO: 122 - DNA, 21 bp, Artificial Sequence
  Synthetic DNA
aaatcattattaatatttgat

SEQ ID NO: 123 - DNA, 21 bp, Artificial Sequence
  Synthetic DNA
aaatcattattaatattagat

SEQ ID NO: 124 - DNA, 22 bp, Artificial Sequence
  Synthetic DNA
cattattaatatttaatmttga

SEQ ID NO: 125 - DNA, 22 bp, Artificial Sequence
  Synthetic DNA
cattattaatatttaatmgatc

SEQ ID NO: 126 - DNA, 36 bp, Artificial Sequence
  Synthetic DNA
ccaattctcatagaaaatatgatagaataaatgtat

SEQ ID NO: 127 - DNA, 36 bp, Artificial Sequence
  Synthetic DNA
ccaattctcatagaaaatatgatagaataaatgcaa

SEQ ID NO: 128 - DNA, 32 bp, Artificial Sequence
  Synthetic DNA
tgattttgaaaggatctgactgtatgtttaca

SEQ ID NO: 129 - DNA, 32 bp, Artificial Sequence
  Synthetic DNA
tgattttgaaaggatctgactgtatgtttatg

SEQ ID NO: 130 - DNA, 500 bp, Stevia rebaudiana
aatcagtccaatttaaacgtgctctacttacagagttatgatatttattaaggcactaaaacatgaaactgacgtgacgaattgaaagattattccaatcttgatccattttgccacttaaaacaagatgaagataacataaaaaagatcggaaaaaaatgataccatgtaaacgaatacgaaacaacataaaacaattaggtacccttgagttttgatttcctggtaaaaactaaataaaaaacacattaattcacaacaaacgattatgaccggtgaagaaaaagattggaacagatgatgaaggaataacatattctcctgatgatcgatgatagatgagaaattggggtattaaggtttgcaattccaaaggaattcgtcagataggagaaactgaaaacagaatatcatgtcttatttaaaaaaaacgggtatgagtttgtgtttgtgggtttttgggttaaatatgaattgagttactctgatgaagagaagtg

SEQ ID NO: 131 - DNA, 39 bp, Artificial Sequence
  Synthetic DNA
aatcagtccaatttaaacgtgctctacttacagagttat

SEQ ID NO: 132 - DNA, 29 bp, Artificial Sequence
  Synthetic DNA
cacttctcttcatcagagtaactcaattc

SEQ ID NO: 133 - DNA, 500 bp, Stevia rebaudiana
aatcagtccaatttaaacgtgctctacttacagagttatcatatttattaaggcactaaaacatgaaactgacgtgacgaattgaaagattattccaatcttgatccattttgccacttaaaacaagatgaagataacataaaaaagatcggaaaaaaatgataccatgtaaacgaatacgaaacaacataaaacaattaggtacccttgagttttgatttcctggtaaaaactaaataaaaaacacattaattcacaacaaacgattatgaccggtgaagaaaaagattggaacagatgatgaaggaataacatattctcctgatgatcgatgatagatgagaaattggggtattaaggtttgcaattccaaaggaattcgtcagataggagaaactgaaaacagaatatcatgtcttatttaaaaaaaacgggtatgagtttgtgtttgtgggtttttgggttaaatatgaattgagttactctgatgaagagaagtg

SEQ ID NO: 134 - DNA, 21 bp, Stevia rebaudiana
acagagttatcatatttatta

SEQ ID NO: 135 - DNA, 41 bp, Stevia rebaudiana
tgctctacttacagagttatcatatttattaaggcactaaa

SEQ ID NO: 136 - DNA, 61 bp, Stevia rebaudiana
aatttaaacgtgctctacttacagagttatcatatttattaaggcactaaaacatgaaact

SEQ ID NO: 137 - DNA, 39 bp, Artificial Sequence
  Synthetic DNA
aatcagtccaatttaaacgtgctctacttacagagatat

SEQ ID NO: 138 - DNA, 29 bp, Artificial Sequence
  Synthetic DNA
cacttctcttcatcagagtaactcaattc

SEQ ID NO: 139 - DNA, 500 bp, Artificial Sequence
  Synthetic DNA
aatcagtccaatttaaacgtgctctacttacagagatatcatatttattaaggcactaaaacatgaaactgacgtgacgaattgaaagattattccaatcttgatccattttgccacttaaaacaagatgaagataacataaaaaagatcggaaaaaaatgataccatgtaaacgaatacgaaacaacataaaacaattaggtacccttgagttttgatttcctggtaaaaactaaataaaaaacacattaattcacaacaaacgattatgaccggtgaagaaaaagattggaacagatgatgaaggaataacatattctcctgatgatcgatgatagatgagaaattggggtattaaggtttgcaattccaaaggaattcgtcagataggagaaactgaaaacagaatatcatgtcttatttaaaaaaaacgggtatgagtttgtgtttgtgggtttttgggttaaatatgaattgagttactctgatgaagagaagtg

SEQ ID NO: 140 - DNA, 500 bp, Artificial Sequence
  Synthetic DNA
aatcagtccaatttaaacgtgctctacttacagagatatgatatttattaaggcactaaaacatgaaactgacgtgacgaattgaaagattattccaatcttgatccattttgccacttaaaacaagatgaagataacataaaaaagatcggaaaaaaatgataccatgtaaacgaatacgaaacaacataaaacaattaggtacccttgagttttgatttcctggtaaaaactaaataaaaaacacattaattcacaacaaacgattatgaccggtgaagaaaaagattggaacagatgatgaaggaataacatattctcctgatgatcgatgatagatgagaaattggggtattaaggtttgcaattccaaaggaattcgtcagataggagaaactgaaaacagaatatcatgtcttatttaaaaaaaacgggtatgagtttgtgtttgtgggtttttgggttaaatatgaattgagttactctgatgaagagaagtg

SEQ ID NO: 141 - DNA, 37 bp, Artificial Sequence
  Synthetic DNA
aatcagtccaatttaaacgtgctctacttacagagat

SEQ ID NO: 142 - DNA, 463 bp, Artificial Sequence
  Synthetic DNA
atcatatttattaaggcactaaaacatgaaactgacgtgacgaattgaaagattattccaatcttgatccattttgccacttaaaacaagatgaagataacataaaaaagatcggaaaaaaatgataccatgtaaacgaatacgaaacaacataaaacaattaggtacccttgagttttgatttcctggtaaaaactaaataaaaaacacattaattcacaacaaacgattatgaccggtgaagaaaaagattggaacagatgatgaaggaataacatattctcctgatgatcgatgatagatgagaaattggggtattaaggtttgcaattccaaaggaattcgtcagataggagaaactgaaaacagaatatcatgtcttatttaaaaaaaacgggtatgagtttgtgtttgtgggtttttgggttaaatatgaattgagttactctgatgaagagaagtg

SEQ ID NO: 143 - DNA, 21 bp, Stevia rebaudiana
acagagttatgatatttatta

SEQ ID NO: 144 - DNA, 41 bp, Stevia rebaudiana
tgctctacttacagagttatgatatttattaaggcactaaa

SEQ ID NO: 145 - DNA, 61 bp, Stevia rebaudiana
aatttaaacgtgctctacttacagagttatgatatttattaaggcactaaaacatgaaact

SEQ ID NO: 146 - DNA, 39 bp, Artificial Sequence
  Synthetic DNA
aatcagtccaatttaaacgtgctctacttacagaggtat

SEQ ID NO: 147 - DNA, 39 bp, Artificial Sequence
  Synthetic DNA
aatcagtccaatttaaacgtgctctacttacagagtgat

SEQ ID NO: 148 - DNA, 39 bp, Artificial Sequence
  Synthetic DNA
aatcagtccaatttaaacgtgctctacttacagagttaa